European Patent Application EP 4 703 387 A1, published March 4, 2026. Title: anti-human CD300A monoclonal antibody and antigen-binding fragment thereof. Applicant: 国立大学法人筑波大学. Application JP. The sequence listing filed with the application follows.

SEQUENCE LISTING (42 sequences)

SEQ ID NO: 1 - protein, 5 aa, Mus musculus
  source 1..5: note = HCDR1 of antibody NO.1
SYGMS

SEQ ID NO: 2 - protein, 17 aa, Mus musculus
  source 1..17: note = HCDR2 of antibody NO.1
TISSGGSYTYYPDSVKG

SEQ ID NO: 3 - protein, 11 aa, Mus musculus
  source 1..11: note = HCDR3 of antibody NO.1
HGDYGYPWFAY

SEQ ID NO: 4 - protein, 12 aa, Mus musculus
  source 1..12: note = LCDR1 of antibody NO.1
TASSSVSSSYLH

SEQ ID NO: 5 - protein, 7 aa, Mus musculus
  source 1..7: note = LCDR2 of antibody NO.1
STSNLAS

SEQ ID NO: 6 - protein, 8 aa, Mus musculus
  source 1..8: note = LCDR3 of antibody NO.1
HQYHRSHT

SEQ ID NO: 7 - protein, 139 aa, Mus musculus
  source 1..139: note = heavy chain variable region of antibody NO.1
MNFGLSLIFLALILKGVQCEVQLVESGGDLVKPGGSLKLSCAASGFTFSSYGMSWVRQTPDKRLEWVATISSGGSYTYYPDSVKGRFTISRDNAKNTLYLQMSSLKSEDTAMYYCARHGDYGYPWFAYWGQGTLVTVSA

SEQ ID NO: 8 - protein, 129 aa, Mus musculus
  source 1..129: note = light chain variable region of antibody NO.1
MDFQVQIFSFLLISASVIMSRGQIVLTQSPAIMSASLGERVTMTCTASSSVSSSYLHWYQQKPGSSPKLWIYSTSNLASGVPARFSGSGSGTSYSLTISSMEAEDAATYYCHQYHRSHTFGGGTKLEIK

SEQ ID NO: 9 - protein, 5 aa, Mus musculus
  source 1..5: note = HCDR1 of antibody NO.2
GYTMN

SEQ ID NO: 10 - protein, 17 aa, Mus musculus
  source 1..17: note = HCDR2 of antibody NO.2
LINPYNGGTSYNQKFKG

SEQ ID NO: 11 - protein, 5 aa, Mus musculus
  source 1..5: note = HCDR3 of antibody NO.2
GAMDY

SEQ ID NO: 12 - protein, 16 aa, Mus musculus
  source 1..16: note = LCDR1 of antibody NO.2
RSSQSLENSNGNTYLN

SEQ ID NO: 13 - protein, 7 aa, Mus musculus
  source 1..7: note = LCDR2 of antibody NO.2
RVSNRFS

SEQ ID NO: 14 - protein, 9 aa, Mus musculus
  source 1..9: note = LCDR3 of antibody NO.2
LQVTHVPWT

SEQ ID NO: 15 - protein, 149 aa, Mus musculus
  source 1..149: note = heavy chain variable region of antibody NO.2
MCPMSSPQTLNTLTPTMGWSWIFLFLLSGTAGVHSEVQLQQSGPELVKPGASMKISCKASGYSFTGYTMNWVKQSHGKNLEWIGLINPYNGGTSYNQKFKGKATLTVDKSSSTAYMELLSLTSEDSAVYYCASGAMDYWGQGTSVTVSS

SEQ ID NO: 16 - protein, 131 aa, Mus musculus
  source 1..131: note = light chain variable region of antibody NO.2
MKLPVRPLVLMFWIPASSSDAVMTQTPLSLPVSLGDQASISCRSSQSLENSNGNTYLNWYLQKPGQSPQLLIYRVSNRFSGVLDRFSGSGSGTDFTLKISRVEAEDLGVYFCLQVTHVPWTFGGGTKLEIK

SEQ ID NO: 17 - protein, 5 aa, Mus musculus
  source 1..5: note = HCDR1 of antibody NO.3
HYGLN

SEQ ID NO: 18 - protein, 17 aa, Mus musculus
  source 1..17: note = HCDR2 of antibody NO.3
WIHTYTGESTYADDFKG

SEQ ID NO: 19 - protein, 8 aa, Mus musculus
  source 1..8: note = HCDR3 of antibody NO.3
GGKDALDY

SEQ ID NO: 20 - protein, 15 aa, Mus musculus
  source 1..15: note = LCDR1 of antibody NO.3
RASESVDNYGISFMN

SEQ ID NO: 21 - protein, 7 aa, Mus musculus
  source 1..7: note = LCDR2 of antibody NO.3
AASNQGS

SEQ ID NO: 22 - protein, 9 aa, Mus musculus
  source 1..9: note = LCDR3 of antibody NO.3
HQSKEVPWT

SEQ ID NO: 23 - protein, 136 aa, Mus musculus
  source 1..136: note = heavy chain variable region of antibody NO.3
MAWVWTLLLLMAAAQSAQAQIQLVQSGPELKKPGETVKISCKASGYTFTHYGLNWVKQAPGKGLQWMGWIHTYTGESTYADDFKGRSAFSLETSASTAYLQINNLKNEDTATYFCARGGKDALDYWGQGTSVTVSS

SEQ ID NO: 24 - protein, 131 aa, Mus musculus
  source 1..131: note = light chain variable region of antibody NO.3
MEKDTLLLWVLLLWVPGSKGDIVLTQSPASLAVSLGQRATISCRASESVDNYGISFMNWFQQKPGQSPKLLIYAASNQGSGVPARFSGSGSGTDFSLNIHPMEEDDIAMYFCHQSKEVPWTFGGGTKLEIK

SEQ ID NO: 25 - protein, 5 aa, synthetic construct
  source 1..5: note = HCDR1 of HuNO.1U
SYGMS

SEQ ID NO: 26 - protein, 17 aa, synthetic construct
  source 1..17: note = HCDR2 of HuNO.1U
TISSGGSYTYYPDSVKG

SEQ ID NO: 27 - protein, 11 aa, synthetic construct
  source 1..11: note = HCDR3 of HuNO.1U
HGDYGYPWFAY

SEQ ID NO: 28 - protein, 12 aa, synthetic construct
  source 1..12: note = LCDR1 of HuNO.1U
TASSSVSSSYLH

SEQ ID NO: 29 - protein, 7 aa, synthetic construct
  source 1..7: note = LCDR2 of HuNO.1U
STSNLAS

SEQ ID NO: 30 - protein, 8 aa, synthetic construct
  source 1..8: note = LCDR3 of HuNO.1U
HQYHRSHT

SEQ ID NO: 31 - protein, 139 aa, synthetic construct
  source 1..139: note = heavy chain variable region of HuNO.1U
MNFGLSLIFLALILKGVQCEVQLVESGGGLVQPGGSLRLSCAASGFTFSSYGMSWVRQAPDKRLEWVATISSGGSYTYYPDSVKGRFTISRDNAKNSLYLQMNSLRAEDTAVYYCARHGDYGYPWFAYWGQGTMVTVSS

SEQ ID NO: 32 - protein, 129 aa, synthetic construct
  source 1..129: note = light chain variable region of HuNO.1U
MDFQVQIFSFLLISASVIMSRGQIQMTQSPSSLSASVGDRVTMTCTASSSVSSSYLHWYQQKPGKAPKLWIYSTSNLASGVPSRFSGSGSGTDYTLTISSLQPEDFATYYCHQYHRSHTFGGGTKVEIK

SEQ ID NO: 33 - DNA, 417 bp, synthetic construct
  source 1..417: mol_type = other DNA; note = heavy chain variable region of HuNO.1U
atgaacttcgggctcagcttgattttccttgccctcattctgaaaggcgtccagtgtgaagtgcagcttgtggagtctgggggaggccttgtgcagcctggagggtccctgagactctcctgtgcagcctctggattcactttcagtagctatggcatgtcttgggttcgccaggctccagacaagaggctggagtgggtcgcaaccattagtagtggaggcagttacacctactatccagacagtgtgaagggacgattcaccatctccagagacaatgccaagaacagcctgtacctgcaaatgaacagtctgagagctgaggacacagccgtgtattactgtgcaagacatggggactatggttacccctggtttgcttactggggccaagggactatggtcactgtctcttca

SEQ ID NO: 34 - DNA, 387 bp, synthetic construct
  source 1..387: mol_type = other DNA; note = light chain variable region of HuNO.1U
atggattttcaggtgcagattttcagcttcctgctcatcagtgcctcagtcatcatgtccagaggacagattcagatgacccagtctccatcatccctgtctgcatctgttggggaccgggtcaccatgacctgcactgccagctcaagtgttagttccagttacttgcactggtaccagcagaagccaggaaaagctcccaaactctggatctatagcacatccaacctggcttctggagtcccatctcgcttcagtggcagtgggtctgggaccgattacactctgacaatcagcagcctgcagcctgaagattttgccacttattactgccaccagtatcatcgttcccacacattcggaggagggaccaaggtggaaatcaaa

SEQ ID NO: 35 - protein, 469 aa, synthetic construct
  source 1..469: note = heavy chain of HuNO.1U
MNFGLSLIFLALILKGVQCEVQLVESGGGLVQPGGSLRLSCAASGFTFSSYGMSWVRQAPDKRLEWVATISSGGSYTYYPDSVKGRFTISRDNAKNSLYLQMNSLRAEDTAVYYCARHGDYGYPWFAYWGQGTMVTVSSASTKGPSVFPLAPSSKSTSGGTAALGCLVKDYFPEPVTVSWNSGALTSGVHTFPAVLQSSGLYSLSSVVTVPSSSLGTQTYICNVNHKPSNTKVDKKVEPKSCDKTHTCPPCPAPEAAGGPSVFLFPPKPKDTLMISRTPEVTCVVVDVSHEDPEVKFNWYVDGVEVHNAKTKPREEQYNSTYRVVSVLTVLHQDWLNGKEYKCKVSNKALPAPIEKTISKAKGQPREPQVYTLPPSRDELTKNQVSLTCLVKGFYPSDIAVEWESNGQPENNYKTTPPVLDSDGSFFLYSKLTVDKSRWQQGNVFSCSVMHEALHNHYTQKSLSLSPGK

SEQ ID NO: 36 - protein, 236 aa, synthetic construct
  source 1..236: note = light chain of HuNO.1U
MDFQVQIFSFLLISASVIMSRGQIQMTQSPSSLSASVGDRVTMTCTASSSVSSSYLHWYQQKPGKAPKLWIYSTSNLASGVPSRFSGSGSGTDYTLTISSLQPEDFATYYCHQYHRSHTFGGGTKVEIKRTVAAPSVFIFPPSDEQLKSGTASVVCLLNNFYPREAKVQWKVDNALQSGNSQESVTEQDSKDSTYSLSSTLTLSKADYEKHKVYACEVTHQGLSSPVTKSFNRGEC

SEQ ID NO: 37 - DNA, 1410 bp, synthetic construct
  source 1..1410: mol_type = other DNA; note = heavy chain of HuNO.1U
atgaacttcgggctcagcttgattttccttgccctcattctgaaaggcgtccagtgtgaagtgcagcttgtggagtctgggggaggccttgtgcagcctggagggtccctgagactctcctgtgcagcctctggattcactttcagtagctatggcatgtcttgggttcgccaggctccagacaagaggctggagtgggtcgcaaccattagtagtggaggcagttacacctactatccagacagtgtgaagggacgattcaccatctccagagacaatgccaagaacagcctgtacctgcaaatgaacagtctgagagctgaggacacagccgtgtattactgtgcaagacatggggactatggttacccctggtttgcttactggggccaagggactatggtcactgtctcttcagcctccaccaagggcccatcggtcttccccctggcaccctcctccaagagcacctctgggggcacagcggccctgggctgcctggtcaaggactacttccccgaaccggtgacggtgtcgtggaactcaggcgccctgaccagcggcgtgcacaccttcccggctgtcctacagtcctcaggactctactccctcagcagcgtggtgaccgtgccctccagcagcttgggcacccagacctacatctgcaacgtgaatcacaagcccagcaacaccaaggtggacaagaaagttgagcccaaatcttgtgacaaaactcacacatgcccaccgtgcccagcacctgaagctgctggaggaccgtcagtcttcctcttccccccaaaacccaaggacaccctcatgatctcccggacccctgaggtcacatgcgtggtggtggacgtgagccacgaagaccctgaggtcaagttcaactggtacgtggacggcgtggaggtgcataatgccaagacaaagccgcgggaggagcagtacaacagcacgtaccgtgtggtcagcgtcctcaccgtcctgcaccaggactggctgaatggcaaggagtacaagtgcaaggtctccaacaaagccctcccagcccccatcgagaaaaccatctccaaagccaaagggcagccccgagaaccacaggtgtacaccctgcccccatcccgggatgagctgaccaagaaccaggtcagcctgacctgcctggtcaaaggcttctatcccagcgacatcgccgtggagtgggagagcaatgggcagccggagaacaactacaagaccacgcctcccgtgctggactccgacggctccttcttcctctacagcaagctcaccgtggacaagagcaggtggcagcaggggaacgtcttctcatgctccgtgatgcatgaggctctgcacaaccactacacgcagaagagcctctccctgtctccgggtaaatga

SEQ ID NO: 38 - DNA, 711 bp, synthetic construct
  source 1..711: mol_type = other DNA; note = light chain of HuNO.1U
atggattttcaggtgcagattttcagcttcctgctcatcagtgcctcagtcatcatgtccagaggacagattcagatgacccagtctccatcatccctgtctgcatctgttggggaccgggtcaccatgacctgcactgccagctcaagtgttagttccagttacttgcactggtaccagcagaagccaggaaaagctcccaaactctggatctatagcacatccaacctggcttctggagtcccatctcgcttcagtggcagtgggtctgggaccgattacactctgacaatcagcagcctgcagcctgaagattttgccacttattactgccaccagtatcatcgttcccacacattcggaggagggaccaaggtggaaatcaaacgaactgtggctgcaccatctgtcttcatcttcccgccatctgatgagcagttgaaatctggaactgcctctgttgtgtgcctgctgaataacttctatcccagagaggccaaagtacagtggaaggtggataacgccctccaatcgggtaactcccaggagagtgtcacagagcaggacagcaaggacagcacctacagcctcagcagcaccctgacgctgagcaaagcagactacgagaaacacaaagtctacgcctgcgaagtcacccatcagggcctgagctcgcccgtcacaaagagcttcaacaggggagagtgttag

SEQ ID NO: 39 - protein, 163 aa, Homo sapiens [sequence omitted]

SEQ ID NO: 40 - protein, 163 aa, Homo sapiens
  source 1..163: note = a part of human CD300A-Q
LSKCRTVAGPVGGSLSVQCPYEKEHRTLNKYWCRPPQIFLCDKIVETKGSAGKRNGRVSIRDSPANLSFTVTLENLTEEDAGTYWCGVDTPWLQDFHDPVVEVEVSVFPASTSMTPASITAAKTSTITTAFPPVSSTTLFAVGATHSASIQEETEEVVNSQLP

SEQ ID NO: 41 - protein, 163 aa, Homo sapiens
  source 1..163: note = a part of human CD300C
GYFPLSHPMTVAGPVGGSLSVQCRYEKEHRTLNKFWCRPPQILRCDKIVETKGSAGKRNGRVSIRDSPANLSFTVTLENLTEEDAGTYWCGVDTPWLRDFHDPIVEVEVSVFPAGTTTASSPQSSMGTSGPPTKLPVHTWPSVTRKDSPEPSPHPGSLFSNVR

SEQ ID NO: 42 - protein, 163 aa, Macaca fascicularis
  source 1..163: note = a part of Macaca fascicularis CD300A
LRGPSTVDGPVGGSLSVQCWYEEEHKTLNKYWCRPPRVLRCAKIVETEGPAGKMNGRVSIMDCPQNLSFTVTLENLTEEDAGTYWCGVDTPWLQDLHDPYVQVEVSVFPASTSMTPTSITAAKTSTITTVFPPVSSTSLFAMSATHSTSNWKENEEVVSSQLP